European Patent Application EP 4 428 231 A1, published September 11, 2024. Title: 고역가 일본뇌염 바이러스 유전형 5형 및 이의 용도. Applicant: 질병관리청. Application KR. The sequence listing filed with the application follows.

SEQUENCE LISTING (1 sequence)

SEQ ID NO: 1 - DNA, 10987 bp, Japanese encephalitis virus
  source 1..10987: mol_type = genomic DNA
tagaagtttatctgtgtgaacttcttggcttagtattgttgagaggaatcgagagattagtgcagtttaaacagttttttagaacggaagaaaaccatgactaaaaaaccaggagggcccggtaaaaaccgggctatcaatatgctgaaacgcggcataccccgcgtatccccacttgtgggggtgaagagggtaattatgaacttgctcgacggcagagggccaatacgattcgttttggctctcttggcgtttttcaatttcacatcactagccccgaccaaggcactcgttagccgatggaaggcagtatagaaaaacgttgcaatgaaacatctcaccagtttcaaaaaggaactgggaacgctcatcaacgctgtaaataagaggggcaaaaaacaaaacaaaagaggaggaagtaatgggacagtcatctggataatgggcttggcagttgtggttgccagtgtgagtgcaatcaagctgtcaaattttcaaggcaaggtgctgatgacaatcaacaacaccgatgtggctgatgtgatcaccattcccacctcaaaagggagtaatagatgttgggtccgagctatagatgtgggacacatgtgcgaggacacaatcacttatgaatgcccaaagcttgacgctggcaacgacccggaggacattgactgctggtgcgacaaacaagccgtgtatgtccagtatggacgttgcactaggaccaggcactccaggagaagtagaagatctgtgtcagtgcaaacccacggagaaagttctttagtgaacaaaaaagaagcctggatggattcgacgaaagccactcggtatctcatgaaaacagagaattggatcatacggaatccaggctatgctcttgtggcagtggcacttggatggatgcttggtagcaacaacggccagcgtgtggtattcacaattctcttgctgttggtcgcacccgcatatagcttcaactgcttaggtatgggaaatcgtgacttcatcgaaggagtcagtggagcgacgtgggtggacctggtgctggaaggagacagttgcctcaccatcatggcgaacgacaaaccaacattggacgtgcgcatgataaacatcgaggccacggaactggctgaggtgcgaacctactgctaccacgccacagtggctgacatctcaacagtggcaagatgccccacgactggagaagcccataacacgaagcgagctgacagcagctatgtctgcaagcaaggctacactgatcgtggatggggaaacggatgtgggttgtttgggaaaggcagcattgacacatgcgctaaatttgtttgcagccacaaggccattggaaagataatccagccagaaaacatcaaatatgaagttggagtgtttgttcatggaaccacaacagcagagaaccacggaaattacacagcccagattggggcttcccaggctgccaagttcaccatcacgcccaatgctccttccatcactctgaagcttggagattacggagaagtcacgatggattgcgagccgcgtagtggatttaatactgaggcattttacgtgctgaccgtagggtctaagtcgttcctagtccaccgcgaatggttcaatgatcttgcgcttccgtggctatctccatctagcacaaattggagaaatagagagatcctgatggagttcgaagaggctcacgcgacaaaacagtctgtcgtcgcgcttggatcacaagagggagccttgcatcaggcattggctggtgccatagtggtggagtactctagctcagtgaagttgacatctggtcacctcaaatgcagactaagaatggagaagttggcgttgaaagggaccacctatggtatgtgcacagagaagttctctttttccaagaatccagctgacactggtcatggtacggttgtcatagaattgcagtacaccggcactgacggaccttgcaagatacccatttcttcggtggccagtctgaatgatttaactccagttggtagattggtgacagtcaatccttttgttgccacatccaccgccaattcgaaggttttggtagaattggaaccaccatttggagattcattcattgttgtcggaagaggagataagcagatcaatcaccattggcacaaggctggcagttcactgggaaaggctttcacgactactttgaaaggagctcagaggctggcagcccttggtgacaccgcttgggactttggatccattggaggggttttcaattccattggtaaggccgtgcaccaagtgtttggaggagctttcagaaccctttttggtggcatgtcctggataacacaaggattgatgggagcgctgctgctgtggatgggtatcaacgcacgagatcggtcgattgcactagcttttcttgctacaggaggtgtgctcttgtttctggccaccaatgtccacgccgataccggctgcgccatcgatataaccagaaaagaaatgaggtgtggtagtggcatatttgtgcacaatgacgtggaggcttgggttgatagatacaagtatctacctgagactcccaagtctttagccaaaatagtccacaaagcacacaaggaaggcatttgtggagtgagatcagtcaccagactggaacaccaaatgtgggaggccgtcagggacgagttaaatgtcttgttgaaggagaatgcggtagatcttagtgtggtggtggacaaaccatcaggaagataccgaccagctccattgcggttggccatgactcaggaaaagtttgagatgggttggaaagcatgggggaagagcattctctttgcgccggaactggccaattccacgtttgtgatcgacggacctgaaaccaaagagtgtccagatgagcgtagagcatggaacagcatgcagattgaggattttgggtttggcattacgtcgactcgagtgtggttgaagatcagggaggagcgcacgaatgaatgtgatggagccatcatcggcacggctgttaaagggaacatggcagtgcacagtgacttgtcatactggattgaaagccatctcaacgacacctggaagctcgagagagctgtgtttggagagataaagtcttgcacttggccagaaacacacacgctctggggagatggtgttgaggaaagtgagttgataattccacacacactcgctggacccaaaagcaagcataacagaagagagggttacaagacacagaatcagggaccatgggacgagagtgagatcactcttgattttgactactgtccagggaccacagtcaccattgctgagggatgtgggaaaagggggccctcaatcaggaccaccactgatagtggaaaattaatcactgattggtgttgcaggagctgcactttgccgccactgaggttcaggacagccagtgggtgctggtatggaatggaaatacggcccatgaagcatgatgaatccacgctcgtgaaatcacaagtcaacgcgtttaatggggagatgattgatccttttcagttgggccttctggtgatgtttctggccacccaggaggtccttcgcaagaaggtggacggccagactgacgattcctgcggttttgggggccctacttgttctgatgcttgggggcatcacctacactgatctagtgagatatgtggtgttggtggctgctgctttcgctgaagctaacaatggaggcgatgtagttcatttggccctgattgccgtatttaaaatccaaccggcattcctagtcatgagcatagcaagaacaaattggacaaaccaggaaaacattgccctagtgctaggagctgctttctttcagatggcctcaacagacctggagtttggtatccatgggctgctaaatgcagcggcgacggcctggatggtagtgcgggcgatcacgtttcccacgacctccaccatcacaatgcccatactagctttgctggcgccaggaatgagagctctccatcttgacacctacagaatctttttgcttatcatcggggtctgtgctctgctgcatgaaaggaggaaaaaccatggcgaagaagaaaggtgctgtccttttgggtctagccctaagttccactgggtggttttcaccagccattatggcagctgggctcatggcgtgcaatccaaacaaaaagagaggatggccagcgacagaatttctgtctgcgattgggttgatgtttgctattgttgggggcctggccgagttggacatcgactctatggcgatacctttcatgttagctgggcttatggcagtgtcatatgtggtatcaggaaaagcaacggacatgtggctagaacgtgcggccgacattagttgggaagtggatgcagcgatcacaggcagcagccgaaggttggacgtcaaactagatgatgatggagatttccaccttattgatgatccaggcgtcccatggaaaatttgggtactgcgcatgtcttgcataggattggcggccttcacaccatgggccatcatcccagcggcttttggatattggctgactttgaaaaccacaaagagaggaggcgttttttgggacacaccatcacccaaagtctacgcaaaaggggacacaaccacaggagtgtacaggataatggctcgagggatctttggcgtctaccaagcaggtgttggagtgatgtatgagaacgtgttccacactctgtggcacacgaccagaggagctgccataatgagtggagaaggaaagttgacgccgtactggggaagcgttaaggaggaccgcataacttatgggggcccatggagattcgatcgaaaatggaatggagtggatgacgtgcaaatgattgtagttgaaccaggaaaagcagctgtaaatgtccaaacaaagccgggagtgtttcggactccacacggagaaattggagctgttagcctggattaccctagtgggacatcgggctcacccatcctggacatcaacggtgatatcattggattgtatgggaacggagttgaacttggagatggctcatatgtgagcgccattgtgcagggtgaacggcaagaagagcccatccccgatgcatacaatccaaacatgctcaagaaaaggcagctgaccgtgttggacttgcatccaggatctgggaaaacaaggaaaatcttaccccaaatcatcaaggatgccattcaacagcgtctcagaacagctgttctggcgcccactcgggttgttgcagctgagatggcagaagctcttagaggacttcccgttagataccaaacttcagcggttccgcgagaacatcaggggaatgagatagttgatgtcatgtgtcacgccaccttaacgcataagctgatgtcaccaaatcgcgtccccaattacaacttgtttgtcatggatgaggcccatttcacagacccagccagcatcgccgctagaggatacatatccaccagagtggaattgggagaagccgcggctatcttcatgactgccactccaccaggaacgactgaccccttccctgactccaacgctcccattcatgatttgcaggacgagatccctgacagagcatggagcagtgggtatgaatggataactgagtactctgggaagacagtatggtttgtggcgagtgtgaaaatgggcaacgaaatcgcagtgtgtctacagagagccggaaagagagtcatccagttaaatcggaaatcttatgacaccgagtaccccaaatgtaagaatggggattgggattttgtcatcaccacggacatttctgaaatgggggccaactttggagcgagcagagtgattgattgtaggaagagtgtgaaacccaccattctggaagaaggagaaggaagagtcattctcagcaacccatcgcctatcaccagtgcgagtgcagcccagcggagaggcagagtgggcagaaatccaaatcaggttggagatgagtaccattacggaggggtcacaagtgaagatgacaccaacctagcacactggacagaagccaagatcatgttggacaacatccacctgccaaatgggttggtagctcagctctatggacctgaaagggaaaaggccttcacaatggacggtgagtatcgattgaggggtgaagaaaagaagaactttctggagttaatcagaacagccgacctccccgtatggctagcttacaaagtggcttcaaatggaatacagtacaccgataggagatggtgttttgatggacctcggacgaatgctatcttagaagacagcactgaagtagagataatcaccagaacgggagaaaggaaaattctaaaaccaagatggctggacgcacgggtgtacgcagatcaccaggctttgaagtggtttaaggacttcgcagcaggaaagagatcagctgtcagttttctagaggtgcttgggcgcatgccagagcacttcatggggaaaacgcgtgaagctcttgatacaatgtacctggttgccacggcagaaaaagggggaaaagctcaccgaatggccctggaggaactgccagatgcactggagacggtgacactcatcgcagcgcttgccgtgatgacaggtgggttctttctactcatgatgcaacgaaagggcataggaaaaatgggcctcggggctctcgtgctcaccctggccactttcttcttgtggatggcagaggtctcagggacgaaaatagccgggaccttactcatagcgttgctgcttatggtggtactcatcccggagccggagaagcaaagatcccaaacggacaaccagttggccgtgtttctgatctgcgtcctcaccgtagtgggaattgtggctgctaatgagtatggcatgctcgaaaagaccaaggaagacataaggaatgtgtttggtaacaaggttcagacatccaatgcacctggaagcctatcaagtctggcgctcgatctacgaccagcaacggcttgggccttatatggaggtagtacagtgattttaactccactgctgaaacatttgatcacctctgagtatgtgacaacatcactagcttcaatcaactcacaggccggctcactttttgttttgccaaaaggcatgcctttcacggatttggatctgacggttggactcgtctttctgggttgttgggggcaaatcactctcaccacttttctgacagctggagtgttagtagttctgcattacggctatatgctccctggctggcaagctgaagccctgagggcagctcagagacgaacagctgcgggtatcatgaagaacgccgttgtggatgggatggttgccactgatgtgcctgaattggaaagaacaacacccctaatgcagaagaaggtggggcaagtgttgctaataggagtcagtatagcagcttttcttgtcaatcccaatgtcaccaccgtgcgagaagccggtgtgctggtgaccgctgctacgctcaccctatgggataatggagcaagtgccgtctggaattcaactacagccacaggactctgccacgtcatgcgaggcagttacttggctggtggttcaatagcttggactctcatcaagaatgttgataaaccatccttgaaaagaggaaggcctggaggaagaacgctgggtgagcaatggaaagaaaaattgaacgccatgaacaaagaagagtttttcaggtacaggaaagaagccatagttgaggtggaccgcacagaggcacgcagggctagacgagagaataacaaagtgggaggtcatcccgtgtcacgaggttcagcaaagctccgatggatggtggagaaagggtttgtctcccctgttggaaaggttgtggaccttggctgtgggcggggaggatggtgctattatgctgccactctgaaaaaagtgcaagaagttaaaggttatacaaaaggaggggccggacatgaggaaccgatgctgatgcaaagctatggttggaatctggtcacgatgaagagtggagtggatgtgttctacagaccttcagagcctagtgacaccctgctctgtgacataggggagtcttctccaagtccagacgtcgaggagcaacgcactctgcgggttctggaaatggcatcagagtggctacaccgaggacccagagaattctgcattaaagttttgtgtccatacatgccaaaggtgatagaaaagatggaaacgctacaacgtcgctttggaggcggactggtgcgcgttcccctgtcacgcaactcaaatcacgaaatgtactgggttagtggggctgctgggaacgtggtacatgctgtaaacatgaccagtcaagttttgctggggcgaatggaccgaccagtctggagaggacccaaatatgaagaagatgtcaacttgggaagcgggaccagagctgtagggaaaggtgaggttcacagtgaccaaggaaaaatcaagaagcggatagagaagctgaaagaagagtatgcagcgacgtggcacgaggaccctgaacatccataccgcacttggacataccatggaagctatgaagtgaaggccaccggttcagccagctcccttgtcaacggagtggttaagctcatgagtaaaccttgggatgccatcactagtgtcaccaccatggccatgactgacactactccctttggtcagcagagagtcttcaaagaaaaagttgacaccaaggcgcctgagccacctgcaggagttcgggaagtgctggacgaaactaccaactggctgtgggcctacttgtcaagagagaaaagacctcgcttgtgtacgagagaggagttcatccggaaagtcaacagcaacgcagctcttggagccatgtttgccgagcaaaatcagtggagctcagccagggaggctgttagtgacccggccttctggaacatggtcgacattgaaagagagaaccacctacgaggggagtgccacacctgcatctacaacatgatgggaaaaagagaaaagaaacctggtgagtttgggaaggctaaaggaagcagagctatctggttcatgtggctcggagcccgctacctggaattcgaggcactcgggttcctgaacgaggaccattggctgagcagggagaactctggaggaggagtggaaggctcaggcatacagaagctagggtacattttgcgagacatctcaacgaaatctggagggaaaatgtatgctgatgacaccgcaggctgggacactaggatcacaagggttgatctggacaatgaggcaaaggtgctggaacttctggatggggagcacaggatgttggcccgtgctattatagaattgacttacaaacacaaagttgtcaaagtaatgaggccagcagtaggtggaaagaccgtgatggatgtgatctctagagaagatcaaagagggagtgggcaagtggtcacatatgctctcaacaccttcacaaacatagctgtccagctagtgaggttgatggaggctgaaggggttgtcggtccacaggatgtggagcagctccccaggaaaaccaaattcgcagtcaggacatggctttttgaaaatggagaagagagagtcaccagaatggcagtgagtggggatgactgcgttgtcaaacctttggatgacagattcgcgcatgctttacacttcttgaatgcgatgtcaaaggtgaggaaagacatacaagaatggaagccatctcaaggctggcacgactggcagcaagtccctttctgctcgaaccactttcaggagattgtgatgaaggatggtagaagccttgttgtgccctgccggggacaggatgagttaataggcagggcccggatttcaccaggagcaggatggaatgtgagagacacagcctgcctagctaaggcctacgcccaaatgtggctcctcctctactttcaccggagagacttgcgccttatggccaacgcgatctgctcagccgttccggtagactgggtacccacaggtaggacatcatggtcgatacactcaaaaggagagtggatgacaacagaagacatgctgcaggtgtggaacagggtatggattgaggagaatgaatggatgagagacaaaacccccgtcgccagttggaccgacgtcccatacgtcggaaagagggaagacatctggtgcggcagcttgatcggaacgcggacaagggccacctgggcagaaaacatctatgcagcaataaaccaagtgagagcaataattggaaatgaaaagtatgtggactacatgacatcacttaggaggtatgaagacactttggtccaggaagatagagtaatttaaaaaacttttggtaatgagtgtaaatagtagtatttattgtaaatagtgtaaataaacaaatttaaataggaagtcaggccgacgtaagtcgccaccggatgctgagtagacggtgctgcctgcgcctcagccccaggaggactgggttaacaaatctgacaaccgaaggtaggaaagccctcaaaaccgtctcggaagaaggtccctgcttactggaggttggaagaccgtgtcaggccacgcaagtgccacttcgctgaggagtgcagcctgtacagccccgggaggaccgggtaaacaaagccgatgaggcccccacggcccaaacctcatccaggatgcaatggatgaggcgtaaggactagaggttagaggagaccccgtggaaaagaaaatgcggcccaaactctttcgaagctgtagaaggagtggaaggactagaggttagaggagaccccgcatttgcatcaaaacagcatattgacacctgggattagactaggagatcttctgatctatctcaacatcagctacaaggcacagagcgccgaaatatgtagctggtggtggggaagaacacaggatct